European Patent Application EP 4 711 384 A1, published March 18, 2026. Title: Antibody binding to il-18 receptor, il-18 receptor activator, and use thereof. Applicant: Wio Bioscience Co., Ltd. Application US. The sequence listing filed with the application follows.

SEQUENCE LISTING (75 sequences)

SEQ ID NO: 1 - protein, 232 aa, synthetic construct
EPKSSDKTHTCPPCPAPEAAGGPSVFLFPPKPKDTLMISRTPEVTCVVVDVSHEDPEVKFNWYVDGVEVHNAKTKPREEQYNSTYRVVSVLTVLHQDWLNGKEYKCKVSNKALPAPIEKTISKAKGQPREPQVYTLPPSRDELTKNQVSLTCLVKGFYPSDIAVEWESNGQPENNYKTTPPVLDSDGSFFLYSKLTVDKSRWQQGNVFSCSVMHEALHNHYTQKSLSLSPGK

SEQ ID NO: 2 - protein, 229 aa, synthetic construct
ASVPRDCGCKPCICTVPEVSSVFIFPPKPKDVLTITLTPKVTCVVVDISKDDPEVQFSWFVDDVEVHTAQTQPREEQFNSTFRSVSELPIMHQDWLNGKEFKCRVNSAAFPAPIEKTISKTKGRPKAPQVYTIPPPKEQMAKDKVSLTCMITDFFPEDITVEWQWNGQPAENYKNTQPIMDTDGSYFVYSKLNVQKSNWEAGNTFTCSVLHEGLHNHHTEKSLSHSPGK

SEQ ID NO: 3 - protein, 232 aa, synthetic construct
ASPTTESKCPKCPAPELLGGPSVFIFPPKPKDVLSISGRPEVTCVVVDVGQEDPEVSFNWYIDGAEVRTANTRPKEEQFNSTYRVVSVLPIQHQDWLTGKEFKCKVNNKALPAPIEKTISKAKGQTREPQVYTLAPHREELAKDTVSVTCLVKGFYPPDINVEWQRNRQPEPEGTYATTPPQLDNDGTYFLYSKLSVGKNTWQRGETFTCVVMHEALHNHYTQKSITQSSGK

SEQ ID NO: 4 - protein, 6 aa, synthetic construct
HHHHHH

SEQ ID NO: 5 - protein, 329 aa, synthetic construct
MNCRELPLTLWVLISVSTAESCTSRPHITVVEGEPFYLKHCSCSLAHEIETTTKSWYKSSGSQEHVELNPRSSSRIALHDCVLEFWPVELNDTGSYFFQMKNYTQKWKLNVIRRNKHSCFTERQVTSKIVEVKKFFQITCENSYYQTLVNSTSLYKNCKKLLLENNKNPTIKKNAEFEDQGYYSCVHFLHHNGKLFNITKTFNITIVEDRSNIVPVLLGPKLNHVAVELGKNVRLNCSALLNEEDVIYWMFGEENGSDPNIHEEKEMRIMTPEGKWHASKVLRIENIGESNLNVLYNCTVASTGGTDTKSFILVRKADMADIPGHVFTR

SEQ ID NO: 6 - protein, 357 aa, synthetic construct
MLCLGWIFLWLVAGERIKGFNISGCSTKKLLWTYSTRSEEEFVLFCDLPEPQKSHFCHRNRLSPKQVPEHLPFMGSNDLSDVQWYQQPSNGDPLEDIRKSYPHIIQDKCTLHFLTPGVNNSGSYICRPKMIKSPYDVACCVKMILEVKPQTNASCEYSASHKQDLLLGSTGSISCPSLSCQSDAQSPAVTWYKNGKLLSVERSNRIVVDEVYDYHQGTYVCDYTQSDTVSSWTVRAVVQVRTIVGDTKLKPDILDPVEDTLEVELGKPLTISCKARFGFERVFNPVIKWYIKDSDLEWEVSVPEAKSIKSTLKDEIIERNIILEKVTQRDLRRKFVCFVQNSIGNTTQSVQLKEKRG

SEQ ID NO: 7 - protein, 122 aa, synthetic construct
QVQLQESGGGPVQAGGSLRLSCSASTTAYDNACMGWFRQAPGKEREGVASIHLRDRTYYADSVKGRFTLSRDGASKTLYLQMNSLKPEDSGTYYCASSNICNGLNLQGNTYWGQGTQVTVSS

SEQ ID NO: 8 - protein, 126 aa, synthetic construct
QVQLQESGGGPVQAEGSLRLSCTASGNLYRDPCMGWFRQAPGKDREGVAAMNTGADSTFYARSVKGRFTISHDNAKNTLYLQMNSVKPEDTAMYYCAASRYCTERTWTWRYDYDYWGQGTQVTVSS

SEQ ID NO: 9 - protein, 120 aa, synthetic construct
QVQLQESGGGSVQAGETLRLSCTASGSTFDEYDMGWYRQAPGNKCELVSTISTIDGSTYYADSVKGRFTISQDNTKNTVYLQMNSLKPEDTGVYYCEADDRGTWDRGGCWGQGTQVTVSS

SEQ ID NO: 10 - protein, 123 aa, synthetic construct
QVQLQESGGGSVQAGETLRLSCTASGFTVHDMGWYRQAPGNECELVSTISSDGSTYYADSVKGRFTISQDNAKNTVYLQMNSLKPEDTAVYYCAADHFTGLQLAECKADFGYWGQGTQVTVSS

SEQ ID NO: 11 - protein, 123 aa, synthetic construct
QVQLQESGGGSVQAGGSLRLSCVASGTTMSMNYMAWFRQAPGKEREGVASIFRSTHYADSVKGRFTIAEDSAKNTVYLQMNSLKPEDTAVYYCAAGRTKPYLTPLAESQYNYWGQGIQVTVSS

SEQ ID NO: 12 - protein, 124 aa, synthetic construct
QVQLQESGGGLVQAGGSLKLSCAASGYTYGPYCMGWFRQFPGKEREGVAAVGGDGRTWYGNSVKGRFTISQDNAKKTLYLQINALKPEDTAMYYCAADFDRTVCSDDIYDYTYRGQGTQVTVSS

SEQ ID NO: 13 - protein, 117 aa, synthetic construct
QVQLQESGGGSVQPGGSLRLSCAASGFTYIPAYMGWFRQAPGKERERVASISSTDGSTTYADSVKGRFTVSQDTAKNTLYLQMNSLKPEDTAMYYCAAYQFGAFRVWGQGTQVTVSS

SEQ ID NO: 14 - protein, 116 aa, synthetic construct
QVQLQESGGGSVQPGGSLRLSCAASGFTYIPAYMGWFRQAPGKERERVASIKTDGSTTYADSVNGRFTIAQDTAKNTLYLQMDSLKPEDTAMYYCAAYQFGAFRVWGQGTQVTVSS

SEQ ID NO: 15 - protein, 5 aa, synthetic construct
GGGGS

SEQ ID NO: 16 - protein, 251 aa, synthetic construct
EVQLVESGGGLVQPGGSLRLSCAASGHAYDNACMGWFRQAPGKEREGVASIHLRDRTYYADSVKGRFTISRDNSKNTLYLQMNSLRAEDTAVYYCASSNICNALNLQGNTYWGQGTLVTVSSGGGGSEVQLLESGGGLVQPGGSLRLSCAASGYTYGPYCMGWFRQAPGKEREGVAAVGGDARTWYGNSVKGRFTISRDNSKNTLYLQMNSLRAEDTAVYYCAADFDRTVCSDDIYDYTYRGQGTLVTVSS

SEQ ID NO: 17 - protein, 10 aa, synthetic construct
GGGGSGGGGS

SEQ ID NO: 18 - protein, 15 aa, synthetic construct
GGGGSGGGGSGGGGS

SEQ ID NO: 19 - protein, 20 aa, synthetic construct
GGGGSGGGGSGGGGSGGGGS

SEQ ID NO: 20 - protein, 122 aa, synthetic construct
EVQLVESGGGLVQPGGSLRLSCAASGTAYDNACMGWFRQAPGKEREGVASIHLRDRTYYADSVKGRFTISRDNSKNTLYLQMNSLRAEDTAVYYCASSNICNALNLQGNTYWGQGTLVTVSS

SEQ ID NO: 21 - protein, 126 aa, synthetic construct
EVQLVESGGGLVQPGGSLRLSCAASGNLYRDPCMGWFRQAPGKDREGVAAMNTGADSTFYARSVKGRFTISRDNAKNTLYLQMNSLRAEDTAVYYCAASRYCTERTYTWRYDYDYWGQGTLVTVSS

SEQ ID NO: 22 - protein, 120 aa, synthetic construct
EVQLVESGGGLVQPGGSLRLSCAASGSTFDEYDMGWYRQAPGGKCELVSTISTIDASTYYADSVKGRFTISRDNSKNTLYLQMNSLRAEDTAVYYCEADDRGTWDRGGCWGQGTLVTVSS

SEQ ID NO: 23 - protein, 123 aa, synthetic construct
EVQLVESGGGLVQPGGSLRLSCAASGFTVHDMGWYRQAPGKECELVSTISSDASTYYADSVKGRFTISRDNAKNTLYLQMNSLRAEDTAVYYCAADSFTGLQLAECKADFGYWGQGTLVTVSS

SEQ ID NO: 24 - protein, 124 aa, synthetic construct
EVQLLESGGGLVQPGGSLRLSCAASGYTYGPYCMGWFRQAPGKEREGVAAVGGDARTWYGNSVKGRFTISRDNSKNTLYLQMNSLRAEDTAVYYCAADFDRTVCSDDIYDYTYRGQGTLVTVSS

SEQ ID NO: 25 - protein, 117 aa, synthetic construct
EVQLVESGGGLVQPGGSLRLSCAASGFTYIPAYMGWFRQAPGKERERVASISSTEGSTTYADSVKGRFTISQDNSKNTLYLQMNSLRPEDTAVYYCAAYQFGAFRVWGQGTLVTVSS

SEQ ID NO: 26 - protein, 116 aa, synthetic construct
EVQLVESGGGLVQPGGSLRLSCAASGFTYIPAYMGWFRQAPGKERERVASIKTDASTTYADSVEGRFTISQDNAKNTLYLQMNSLRPEDTAVYYCAAYQFGAFRVWGQGTLVTVSS

SEQ ID NO: 27 - protein, 5 aa, synthetic construct
NACMG

SEQ ID NO: 28 - protein, 16 aa, synthetic construct
SIHLRDRTYYADSVKG

SEQ ID NO: 29 - protein, 14 aa, synthetic construct
SNICNGLNLQGNTY

SEQ ID NO: 30 - protein, 5 aa, synthetic construct
DPCMG

SEQ ID NO: 31 - protein, 17 aa, synthetic construct
AMNTGADSTFYARSVKG

SEQ ID NO: 32 - protein, 17 aa, synthetic construct
SRYCTERTWTWRYDYDY

SEQ ID NO: 33 - protein, 5 aa, synthetic construct
EYDMG

SEQ ID NO: 34 - protein, 17 aa, synthetic construct
TISTIDGSTYYADSVKG

SEQ ID NO: 35 - protein, 11 aa, synthetic construct
DDRGTWDRGGC

SEQ ID NO: 36 - protein, 5 aa, synthetic construct
VHDMG

SEQ ID NO: 37 - protein, 16 aa, synthetic construct
TISSDGSTYYADSVKG

SEQ ID NO: 38 - protein, 17 aa, synthetic construct
DHFTGLQLAECKADFGY

SEQ ID NO: 39 - protein, 5 aa, synthetic construct
MNYMA

SEQ ID NO: 40 - protein, 14 aa, synthetic construct
SIFRSTHYADSVKG

SEQ ID NO: 41 - protein, 17 aa, synthetic construct
GRTKPYLTPLAESQYNY

SEQ ID NO: 42 - protein, 5 aa, synthetic construct
PYCMG

SEQ ID NO: 43 - protein, 16 aa, synthetic construct
AVGGDGRTWYGNSVKG

SEQ ID NO: 44 - protein, 16 aa, synthetic construct
DFDRTVCSDDIYDYTY

SEQ ID NO: 45 - protein, 5 aa, synthetic construct
PAYMG

SEQ ID NO: 46 - protein, 16 aa, synthetic construct
ISSTDGSTTYADSVKG

SEQ ID NO: 47 - protein, 8 aa, synthetic construct
YQFGAFRV

SEQ ID NO: 48 - protein, 5 aa, synthetic construct
PAYMG

SEQ ID NO: 49 - protein, 15 aa, synthetic construct
IKTDGSTTYADSVNG

SEQ ID NO: 50 - protein, 8 aa, synthetic construct
YQFGAFRV

SEQ ID NO: 51 - protein, 14 aa, synthetic construct
SNICNALNLQGNTY

SEQ ID NO: 52 - protein, 17 aa, synthetic construct
SRYCTERTYTWRYDYDY

SEQ ID NO: 53 - protein, 17 aa, synthetic construct
TISTIDASTYYADSVKG

SEQ ID NO: 54 - protein, 16 aa, synthetic construct
TISSDASTYYADSVKG

SEQ ID NO: 55 - protein, 17 aa, synthetic construct
DSFTGLQLAECKADFGY

SEQ ID NO: 56 - protein, 15 aa, synthetic construct
VGGDARTWYGNSVKG

SEQ ID NO: 57 - protein, 16 aa, synthetic construct
ISSTEGSTTYADSVKG

SEQ ID NO: 58 - protein, 15 aa, synthetic construct
IKTDASTTYADSVEG

SEQ ID NO: 59 - protein, 251 aa, synthetic construct
EVQLVESGGGLVQPGGSLRLSCAASGTAYDNACMGWFRQAPGKEREGVASIHLRDRTYYADSVKGRFTISRDNSKNTLYLQMNSLRAEDTAVYYCASSNICNALNLQGNTYWGQGTLVTVSSGGGGSEVQLLESGGGLVQPGGSLRLSCAASGYTYGPYCMGWFRQAPGKEREGVAAVGGDARTWYGNSVKGRFTISRDNSKNTLYLQMNSLRAEDTAVYYCAADFDRTVCSDDIYDYTYRGQGTLVTVSS

SEQ ID NO: 60 - protein, 247 aa, synthetic construct
EVQLVESGGGLVQPGGSLRLSCAASGNLYRDPCMGWFRQAPGKDREGVAAMNTGADSTFYARSVKGRFTISRDNAKNTLYLQMNSLRAEDTAVYYCAASRYCTERTYTWRYDYDYWGQGTLVTVSSGGGGSEVQLVESGGGLVQPGGSLRLSCAASGFTYIPAYMGWFRQAPGKERERVASIKTDASTTYADSVEGRFTISQDNAKNTLYLQMNSLRPEDTAVYYCAAYQFGAFRVWGQGTLVTVSS

SEQ ID NO: 61 - protein, 248 aa, synthetic construct
EVQLVESGGGLVQPGGSLRLSCAASGNLYRDPCMGWFRQAPGKDREGVAAMNTGADSTFYARSVKGRFTISRDNAKNTLYLQMNSLRAEDTAVYYCAASRYCTERTYTWRYDYDYWGQGTLVTVSSGGGGSEVQLVESGGGLVQPGGSLRLSCAASGFTYIPAYMGWFRQAPGKERERVASISSTEGSTTYADSVKGRFTISQDNSKNTLYLQMNSLRPEDTAVYYCAAYQFGAFRVWGQGTLVTVSS

SEQ ID NO: 62 - protein, 245 aa, synthetic construct
EVQLVESGGGLVQPGGSLRLSCAASGFTVHDMGWYRQAPGKECELVSTISSDASTYYADSVKGRFTISRDNAKNTLYLQMNSLRAEDTAVYYCAADSFTGLQLAECKADFGYWGQGTLVTVSSGGGGSEVQLVESGGGLVQPGGSLRLSCAASGFTYIPAYMGWFRQAPGKERERVASISSTEGSTTYADSVKGRFTISQDNSKNTLYLQMNSLRPEDTAVYYCAAYQFGAFRVWGQGTLVTVSS

SEQ ID NO: 63 - protein, 251 aa, synthetic construct
QVQLQESGGGPVQAGGSLRLSCSASTTAYDNACMGWFRQAPGKEREGVASIHLRDRTYYADSVKGRFTLSRDGASKTLYLQMNSLKPEDSGTYYCASSNICNGLNLQGNTYWGQGTQVTVSSGGGGSQVQLQESGGGLVQAGGSLKLSCAASGYTYGPYCMGWFRQFPGKEREGVAAVGGDGRTWYGNSVKGRFTISQDNAKKTLYLQINALKPEDTAMYYCAADFDRTVCSDDIYDYTYRGQGTQVTVSS

SEQ ID NO: 64 - protein, 244 aa, synthetic construct
QVQLQESGGGPVQAEGSLRLSCTASGNLYRDPCMGWFRQAPGKDREGVAAMNTGADSTFYARSVKGRFTISHDNAKNTLYLQMNSVKPEDTAMYYCAASRYCTERTWTWRYDYDYWGQGTQVTVSSGSQVQLQESGGGSVQPGGSLRLSCAASGFTYIPAYMGWFRQAPGKERERVASIKTDGSTTYADSVNGRFTIAQDTAKNTLYLQMDSLKPEDTAMYYCAAYQFGAFRVWGQGTQVTVSS

SEQ ID NO: 65 - protein, 483 aa, synthetic construct
QVQLQESGGGPVQAGGSLRLSCSASTTAYDNACMGWFRQAPGKEREGVASIHLRDRTYYADSVKGRFTLSRDGASKTLYLQMNSLKPEDSGTYYCASSNICNGLNLQGNTYWGQGTQVTVSSGGGGSQVQLQESGGGLVQAGGSLKLSCAASGYTYGPYCMGWFRQFPGKEREGVAAVGGDGRTWYGNSVKGRFTISQDNAKKTLYLQINALKPEDTAMYYCAADFDRTVCSDDIYDYTYRGQGTQVTVSSEPKSSDKTHTCPPCPAPEAAGGPSVFLFPPKPKDTLMISRTPEVTCVVVDVSHEDPEVKFNWYVDGVEVHNAKTKPREEQYNSTYRVVSVLTVLHQDWLNGKEYKCKVSNKALPAPIEKTISKAKGQPREPQVYTLPPSRDELTKNQVSLTCLVKGFYPSDIAVEWESNGQPENNYKTTPPVLDSDGSFFLYSKLTVDKSRWQQGNVFSCSVMHEALHNHYTQKSLSLSPGK

SEQ ID NO: 66 - protein, 6 aa, synthetic construct
GGGGSG

SEQ ID NO: 67 - protein, 6 aa, synthetic construct
GGGSGG

SEQ ID NO: 68 - protein, 6 aa, synthetic construct
GGSGGG

SEQ ID NO: 69 - protein, 6 aa, synthetic construct
GSGGGG

SEQ ID NO: 70 - protein, 6 aa, synthetic construct
GGSGSG

SEQ ID NO: 71 - protein, 6 aa, synthetic construct
GSGSGG

SEQ ID NO: 72 - protein, 478 aa, synthetic construct
EVQLVESGGGLVQPGGSLRLSCAASGFTVHDMGWYRQAPGKECELVSTISSDASTYYADSVKGRFTISRDNAKNTLYLQMNSLRAEDTAVYYCAADSFTGLQLAECKADFGYWGQGTLVTVSSGGGGSGEVQLVESGGGLVQPGGSLRLSCAASGFTYIPAYMGWFRQAPGKERERVASISSTEGSTTYADSVKGRFTISQDNSKNTLYLQMNSLRPEDTAVYYCAAYQFGAFRVWGQGTLVTVSSEPKSSDKTHTCPPCPAPEAAGGPSVFLFPPKPKDTLMISRTPEVTCVVVDVSHEDPEVKFNWYVDGVEVHNAKTKPREEQYNSTYRVVSVLTVLHQDWLNGKEYKCKVSNKALPAPIEKTISKAKGQPREPQVYTLPPSRDELTKNQVSLTCLVKGFYPSDIAVEWESNGQPENNYKTTPPVLDSDGSFFLYSKLTVDKSRWQQGNVFSCSVMHEALHNHYTQKSLSLSPGK

SEQ ID NO: 73 - protein, 478 aa, synthetic construct
EVQLVESGGGLVQPGGSLRLSCAASGFTVHDMGWYRQAPGKECELVSTISSHASTYYADSVKGRFTISRDNAKNTLYLQMNSLRAEDTAVYYCAADSFTGLQLAHCKADFGYWGQGTLVTVSSGGGGSGEVQLVESGGGLVQPGGSLRLSCAASGFTYIPAYMGWFRQAPGKERERVASISSTEGSTTYADSVKGRFTISQDNSKNTLYLQMNSLRPEDTAVYYCAAYQFGAFRVWGQGTLVTVSSEPKSSDKTHTCPPCPAPEAAGGPSVFLFPPKPKDTLMISRTPEVTCVVVDVSHEDPEVKFNWYVDGVEVHNAKTKPREEQYNSTYRVVSVLTVLHQDWLNGKEYKCKVSNKALPAPIEKTISKAKGQPREPQVYTLPPSRDELTKNQVSLTCLVKGFYPSDIAVEWESNGQPENNYKTTPPVLDSDGSFFLYSKLTVDKSRWQQGNVFSCSVMHEALHNHYTQKSLSLSPGK

SEQ ID NO: 74 - protein, 478 aa, synthetic construct
EVQLVESGGGLVQPGGSLRLSCAASGFTVHDMGWYRQAPGKECELVSTISSDASTYYAHSVKGRFTISRDNAKNTLYLQMNSLRAEDTAVYYCAADSFTGLQLAECKAHFGYWGQGTLVTVSSGGGGSGEVQLVESGGGLVQPGGSLRLSCAASGFTYIPAYMGWFRQAPGKERERVASISSTEGSTTYADSVKGRFTISQDNSKNTLYLQMNSLRPEDTAVYYCAAYQFGAFRVWGQGTLVTVSSEPKSSDKTHTCPPCPAPEAAGGPSVFLFPPKPKDTLMISRTPEVTCVVVDVSHEDPEVKFNWYVDGVEVHNAKTKPREEQYNSTYRVVSVLTVLHQDWLNGKEYKCKVSNKALPAPIEKTISKAKGQPREPQVYTLPPSRDELTKNQVSLTCLVKGFYPSDIAVEWESNGQPENNYKTTPPVLDSDGSFFLYSKLTVDKSRWQQGNVFSCSVMHEALHNHYTQKSLSLSPGK

SEQ ID NO: 75 - protein, 478 aa, synthetic construct
EVQLVESGGGLVQPGGSLRLSCAASGFTVHDMGWYRQAPGKECELVSTISSDASTYYADSVKGRFTISRDNAKNTLYLQMNSLRAEDTAVYYCAADSFHGLQLAECKADFGYWGQGTLVTVSSGGGGSGEVQLVESGGGLVQPGGSLRLSCAASGFTYIPAYMGWFRQAPGKERERVASISSTEGSTTYADSVKGRFTISQDNSKNTLYLQMNSLRPEDTAVYYCAAYQFGAFRVWGQGTLVTVSSEPKSSDKTHTCPPCPAPEAAGGPSVFLFPPKPKDTLMISRTPEVTCVVVDVSHEDPEVKFNWYVDGVEVHNAKTKPREEQYNSTYRVVSVLTVLHQDWLNGKEYKCKVSNKALPAPIEKTISKAKGQPREPQVYTLPPSRDELTKNQVSLTCLVKGFYPSDIAVEWESNGQPENNYKTTPPVLDSDGSFFLYSKLTVDKSRWQQGNVFSCSVMHEALHNHYTQKSLSLSPGK